European Patent Application EP 4 186 916 A1, published May 31, 2023. Title: A peptide and use thereof. Applicant: 3HBio. The sequence listing filed with the application follows.

SEQUENCE LISTING (309 sequences)

SEQ ID NO: 1 - protein, 11 aa, Artificial Sequence
  Artificial Sequence
  MISC_FEATURE (1)..(11): 2nd amino acid(Xaa) is L-cyclohexylalanins.
KXVAAWTLKAA

SEQ ID NO: 2 - protein, 13 aa, Artificial Sequence
  Artificial Sequence
PKYVKQNTLKLAT

SEQ ID NO: 3 - protein, 15 aa, Artificial Sequence
  Artificial Sequence
ILMQYIKANSKFIGI

SEQ ID NO: 4 - protein, 15 aa, Artificial Sequence
  Artificial Sequence
QSIALSSLMVAQAIP

SEQ ID NO: 5 - protein, 32 aa, Artificial Sequence
  Artificial Sequence
ILMQYIKANSKFIGIPMGLPQSIALSSLMVAQ

SEQ ID NO: 6 - protein, 15 aa, Artificial Sequence
  Artificial Sequence
RNVPPIFNDVYWIAF

SEQ ID NO: 7 - protein, 15 aa, Artificial Sequence
  Artificial Sequence
CRFRGLISLSQVYLS

SEQ ID NO: 8 - protein, 20 aa, Artificial Sequence
  Artificial Sequence
KTTKQSFDLSVKAQYKKNKH

SEQ ID NO: 9 - protein, 11 aa, Artificial Sequence
  Artificial Sequence
RNVPPIFNDVY

SEQ ID NO: 10 - protein, 11 aa, Artificial Sequence
  Artificial Sequence
CRFRGLISLSQ

SEQ ID NO: 11 - protein, 12 aa, Artificial Sequence
  Artificial Sequence
KTTKQSFDLSVK

SEQ ID NO: 12 - protein, 12 aa, Artificial Sequence
  Artificial Sequence
RNVPPIFNDVYW

SEQ ID NO: 13 - protein, 12 aa, Artificial Sequence
  Artificial Sequence
CRFRGLISLSQV

SEQ ID NO: 14 - protein, 17 aa, Artificial Sequence
  Artificial Sequence
KTTKQSFDLSVKAQYKK

SEQ ID NO: 15 - protein, 13 aa, Artificial Sequence
  Artificial Sequence
RNVPPIFNDVYWI

SEQ ID NO: 16 - protein, 13 aa, Artificial Sequence
  Artificial Sequence
CRFRGLISLSQVY

SEQ ID NO: 17 - protein, 18 aa, Artificial Sequence
  Artificial Sequence
KTTKQSFDLSVKAQYKKN

SEQ ID NO: 18 - protein, 11 aa, Artificial Sequence
  Artificial Sequence
PIFNDVYWIAF

SEQ ID NO: 19 - protein, 11 aa, Artificial Sequence
  Artificial Sequence
GLISLSQVYLS

SEQ ID NO: 20 - protein, 16 aa, Artificial Sequence
  Artificial Sequence
QSFDLSVKAQYKKNKH

SEQ ID NO: 21 - protein, 12 aa, Artificial Sequence
  Artificial Sequence
PPIFNDVYWIAF

SEQ ID NO: 22 - protein, 12 aa, Artificial Sequence
  Artificial Sequence
RGLISLSQVYLS

SEQ ID NO: 23 - protein, 17 aa, Artificial Sequence
  Artificial Sequence
KQSFDLSVKAQYKKNKH

SEQ ID NO: 24 - protein, 13 aa, Artificial Sequence
  Artificial Sequence
VPPIFNDVYWIAF

SEQ ID NO: 25 - protein, 13 aa, Artificial Sequence
  Artificial Sequence
FRGLISLSQVYLS

SEQ ID NO: 26 - protein, 18 aa, Artificial Sequence
  Artificial Sequence
TKQSFDLSVKAQYKKNKH

SEQ ID NO: 27 - protein, 13 aa, Artificial Sequence
  Artificial Sequence
NVPPIFNDVYWIA

SEQ ID NO: 28 - protein, 13 aa, Artificial Sequence
  Artificial Sequence
RFRGLISLSQVYL

SEQ ID NO: 29 - protein, 16 aa, Artificial Sequence
  Artificial Sequence
TKQSFDLSVKAQYKKN

SEQ ID NO: 30 - protein, 11 aa, Artificial Sequence
  Artificial Sequence
VPPIFNDVYWI

SEQ ID NO: 31 - protein, 11 aa, Artificial Sequence
  Artificial Sequence
FRGLISLSQVY

SEQ ID NO: 32 - protein, 16 aa, Artificial Sequence
  Artificial Sequence
TKQSFDLSVKAQYKKN

SEQ ID NO: 33 - protein, 9 aa, Artificial Sequence
  Artificial Sequence
PPIFNDVYW

SEQ ID NO: 34 - protein, 9 aa, Artificial Sequence
  Artificial Sequence
RGLISLSQV

SEQ ID NO: 35 - protein, 14 aa, Artificial Sequence
  Artificial Sequence
KQSFDLSVKAQYKK

SEQ ID NO: 36 - protein, 4 aa, Artificial Sequence
  Artificial Sequence
  MISC_FEATURE (1)..(4): 1st amino acid(Xaa) is a 6-aminohexanoic acid.
XRNV

SEQ ID NO: 37 - protein, 4 aa, Artificial Sequence
  Artificial Sequence
  MISC_FEATURE (1)..(4): 1st amino acid(Xaa) is a D-form alanine. 2nd amino acid(Xaa) is a 6-aminohexanoic acid.
XXRN

SEQ ID NO: 38 - protein, 4 aa, Artificial Sequence
  Artificial Sequence
  MISC_FEATURE (1)..(4): 4th amino acid(Xaa) is a 6-aminohexanoic acid.
IAFX

SEQ ID NO: 39 - protein, 4 aa, Artificial Sequence
  Artificial Sequence
  MISC_FEATURE (1)..(4): 3rd amino acid(Xaa) is a 6-aminohexanoic acid. 4th amino acid(Xaa) is a D-form alanine.
AFXX

SEQ ID NO: 40 - protein, 4 aa, Artificial Sequence
  Artificial Sequence
RNVP

SEQ ID NO: 41 - protein, 4 aa, Artificial Sequence
  Artificial Sequence
WIAF

SEQ ID NO: 42 - protein, 4 aa, Artificial Sequence
  Artificial Sequence
  MISC_FEATURE (1)..(4): 1st amino acid(Xaa) is a 6-aminohexanoic acid.
XCRF

SEQ ID NO: 43 - protein, 4 aa, Artificial Sequence
  Artificial Sequence
  MISC_FEATURE (1)..(4): 1st amino acid(Xaa) is a D-form alanine. 2nd amino acid(Xaa) is a 6-aminohexanoic acid.
XXCR

SEQ ID NO: 44 - protein, 4 aa, Artificial Sequence
  Artificial Sequence
  MISC_FEATURE (1)..(4): 4th amino acid(Xaa) is a 6-aminohexanoic acid.
YLSX

SEQ ID NO: 45 - protein, 4 aa, Artificial Sequence
  Artificial Sequence
  MISC_FEATURE (1)..(4): 3rd amino acid(Xaa) is a 6-aminohexanoic acid. 4th amino acid(Xaa) is a D-form alanine.
LSXX

SEQ ID NO: 46 - protein, 4 aa, Artificial Sequence
  Artificial Sequence
CRFR

SEQ ID NO: 47 - protein, 4 aa, Artificial Sequence
  Artificial Sequence
VYLS

SEQ ID NO: 48 - protein, 4 aa, Artificial Sequence
  Artificial Sequence
  MISC_FEATURE (1)..(4): 1st amino acid(Xaa) is a 6-aminohexanoic acid.
XKTT

SEQ ID NO: 49 - protein, 4 aa, Artificial Sequence
  Artificial Sequence
  MISC_FEATURE (1)..(4): 1st amino acid(Xaa) is a D-form alanine. 2nd amino acid(Xaa) is a 6-aminohexanoic acid.
XXKT

SEQ ID NO: 50 - protein, 4 aa, Artificial Sequence
  Artificial Sequence
  MISC_FEATURE (1)..(4): 4th amino acid(Xaa) is a 6-aminohexanoic acid.
NKHX

SEQ ID NO: 51 - protein, 4 aa, Artificial Sequence
  Artificial Sequence
  MISC_FEATURE (1)..(4): 3rd amino acid(Xaa) is a 6-aminohexanoic acid. 4th amino acid(Xaa) is a D-form alanine.
KHXX

SEQ ID NO: 52 - protein, 15 aa, Artificial Sequence
  Artificial Sequence
GSHHHHHHGSDDDDK

SEQ ID NO: 53 - protein, 6 aa, Artificial Sequence
  Artificial Sequence
HHHHHH

SEQ ID NO: 54 - protein, 20 aa, Artificial Sequence
  Artificial Sequence
MRGSHHHHHHGSDDDDKIVD

SEQ ID NO: 55 - protein, 13 aa, Artificial Sequence
  Artificial Sequence
GGGGSGGGGGGSS

SEQ ID NO: 56 - protein, 30 aa, Artificial Sequence
  Artificial Sequence
  MISC_FEATURE (1)..(30): 16th amino acid(Xaa) is a 6-aminohexanoic acid. 17th amino acid(Xaa) is a D-form alanine. 19th amino acid(Xaa) is L-cyclohexylalanins. 29th amino acid(Xaa) is a D-form alanine. 30th amino acid(Xaa) is a 6-aminohexanoic acid.
RNVPPIFNDVYWIAFXXKXVAAWTLKAAXX

SEQ ID NO: 57 - protein, 30 aa, Artificial Sequence
  Artificial Sequence
  MISC_FEATURE (1)..(30): 1st amino acid(Xaa) is a 6-aminohexanoic acid. 2nd amino acid(Xaa) is a D-form alanine. 4th amino acid(Xaa) is L-cyclohexylalanins. 14th amino acid(Xaa) is a D-form alanine. 15th amino acid(Xaa) is a 6-aminohexanoic acid.
XXKXVAAWTLKAAXXRNVPPIFNDVYWIAF

SEQ ID NO: 58 - protein, 30 aa, Artificial Sequence
  Artificial Sequence
  MISC_FEATURE (1)..(30): 16th amino acid(Xaa) is a 6-aminohexanoic acid. 17th amino acid(Xaa) is a D-form alanine. 19th amino acid(Xaa) is L-cyclohexylalanins. 29th amino acid(Xaa) is a D-form alanine. 30th amino acid(Xaa) is a 6-aminohexanoic acid.
CRFRGLISLSQVYLSXXKXVAAWTLKAAXX

SEQ ID NO: 59 - protein, 30 aa, Artificial Sequence
  Artificial Sequence
  MISC_FEATURE (1)..(30): 1st amino acid(Xaa) is a 6-aminohexanoic acid. 2nd amino acid(Xaa) is a D-form alanine. 4th amino acid(Xaa) is L-cyclohexylalanins. 14th amino acid(Xaa) is a D-form alanine. 15th amino acid(Xaa) is a 6-aminohexanoic acid.
XXKXVAAWTLKAAXXCRFRGLISLSQVYLS

SEQ ID NO: 60 - protein, 35 aa, Artificial Sequence
  Artificial Sequence
  MISC_FEATURE (1)..(35): 21st amino acid(Xaa) is a 6-aminohexanoic acid. 22nd amino acid(Xaa) is a D-form alanine. 24th amino acid(Xaa) is L-cyclohexylalanins. 34th amino acid(Xaa) is a D-form alanine. 35th amino acid(Xaa) is a 6-aminohexanoic acid.
KTTKQSFDLSVKAQYKKNKHXXKXVAAWTLKAAXX

SEQ ID NO: 61 - protein, 35 aa, Artificial Sequence
  Artificial Sequence
  MISC_FEATURE (1)..(35): 1st amino acid(Xaa) is a 6-aminohexanoic acid. 2nd amino acid(Xaa) is a D-form alanine. 4th amino acid(Xaa) is L-cyclohexylalanins. 14th amino acid(Xaa) is a D-form alanine. 15th amino acid(Xaa) is a 6-aminohexanoic acid.
XXKXVAAWTLKAAXXKTTKQSFDLSVKAQYKKNKH

SEQ ID NO: 62 - protein, 26 aa, Artificial Sequence
  Artificial Sequence
  MISC_FEATURE (1)..(26): 17th amino acid(Xaa) is L-cyclohexylalanins.
RNVPPIFNDVYWIAFKXVAAWTLKAA

SEQ ID NO: 63 - protein, 26 aa, Artificial Sequence
  Artificial Sequence
  MISC_FEATURE (1)..(26): 2nd amino acid(Xaa) is L-cyclohexylalanins.
KXVAAWTLKAARNVPPIFNDVYWIAF

SEQ ID NO: 64 - protein, 22 aa, Artificial Sequence
  Artificial Sequence
  MISC_FEATURE (1)..(22): 13rd amino acid(Xaa) is L-cyclohexylalanins.
RNVPPIFNDVYKXVAAWTLKAA

SEQ ID NO: 65 - protein, 22 aa, Artificial Sequence
  Artificial Sequence
  MISC_FEATURE (1)..(22): 13rd amino acid(Xaa) is L-cyclohexylalanins.
PIFNDVYWIAFKXVAAWTLKAA

SEQ ID NO: 66 - protein, 20 aa, Artificial Sequence
  Artificial Sequence
  MISC_FEATURE (1)..(20): 11st amino acid(Xaa) is L-cyclohexylalanins.
PPIFNDVYWKXVAAWTLKAA

SEQ ID NO: 67 - protein, 32 aa, Artificial Sequence
  Artificial Sequence
  MISC_FEATURE (1)..(32): 17th amino acid(Xaa) is L-cyclohexylalanins.
RNVPPIFNDVYWIAFKXVAAWTLKAAHHHHHH

SEQ ID NO: 68 - protein, 45 aa, Artificial Sequence
  Artificial Sequence
  MISC_FEATURE (1)..(45): 16th amino acid(Xaa) is a 6-aminohexanoic acid. 17th amino acid(Xaa) is a D-form alanine. 19th amino acid(Xaa) is L-cyclohexylalanins. 29th amino acid(Xaa) is a D-form alanine. 30th amino acid(Xaa) is a 6-aminohexanoic acid.
RNVPPIFNDVYWIAFXXKXVAAWTLKAAXXGSHHHHHHGSDDDDK

SEQ ID NO: 69 - protein, 45 aa, Artificial Sequence
  Artificial Sequence
  MISC_FEATURE (1)..(45): 16th amino acid(Xaa) is a 6-aminohexanoic acid. 17th amino acid(Xaa) is a D-form alanine. 19th amino acid(Xaa) is L-cyclohexylalanins. 29th amino acid(Xaa) is a D-form alanine. 30th amino acid(Xaa) is a 6-aminohexanoic acid.
GSHHHHHHGSDDDDKXXKXVAAWTLKAAXXRNVPPIFNDVYWIAF

SEQ ID NO: 70 - protein, 45 aa, Artificial Sequence
  Artificial Sequence
  MISC_FEATURE (1)..(45): 31st amino acid(Xaa) is a 6-aminohexanoic acid. 32nd amino acid(Xaa) is a D-form alanine. 34th amino acid(Xaa) is L-cyclohexylalanins. 44th amino acid(Xaa) is a D-form alanine. 45th amino acid(Xaa) is a 6-aminohexanoic acid.
RNVPPIFNDVYWIAFGSHHHHHHGSDDDDKXXKXVAAWTLKAAXX

SEQ ID NO: 71 - protein, 45 aa, Artificial Sequence
  Artificial Sequence
  MISC_FEATURE (1)..(45): 16th amino acid(Xaa) is a 6-aminohexanoic acid. 17th amino acid(Xaa) is a D-form alanine. 19th amino acid(Xaa) is L-cyclohexylalanins. 29th amino acid(Xaa) is a D-form alanine. 30th amino acid(Xaa) is a 6-aminohexanoic acid.
GSHHHHHHGSDDDDKXXKXVAAWTLKAAXXCRFRGLISLSQVYLS

SEQ ID NO: 72 - protein, 45 aa, Artificial Sequence
  Artificial Sequence
  MISC_FEATURE (1)..(45): 31st amino acid(Xaa) is a 6-aminohexanoic acid. 32nd amino acid(Xaa) is a D-form alanine. 34th amino acid(Xaa) is L-cyclohexylalanins. 44th amino acid(Xaa) is a D-form alanine. 45th amino acid(Xaa) is a 6-aminohexanoic acid.
GSHHHHHHGSDDDDKCRFRGLISLSQVYLSXXKXVAAWTLKAAXX

SEQ ID NO: 73 - protein, 45 aa, Artificial Sequence
  Artificial Sequence
  MISC_FEATURE (1)..(45): 16th amino acid(Xaa) is a 6-aminohexanoic acid. 17th amino acid(Xaa) is a D-form alanine. 19th amino acid(Xaa) is L-cyclohexylalanins. 29th amino acid(Xaa) is a D-form alanine. 30th amino acid(Xaa) is a 6-aminohexanoic acid.
CRFRGLISLSQVYLSXXKXVAAWTLKAAXXGSHHHHHHGSDDDDK

SEQ ID NO: 74 - protein, 50 aa, Artificial Sequence
  Artificial Sequence
  MISC_FEATURE (1)..(50): 16th amino acid(Xaa) is a 6-aminohexanoic acid. 17th amino acid(Xaa) is a D-form alanine. 19th amino acid(Xaa) is L-cyclohexylalanins. 29th amino acid(Xaa) is a D-form alanine. 30th amino acid(Xaa) is a 6-aminohexanoic acid.
GSHHHHHHGSDDDDKXXKXVAAWTLKAAXXKTTKQSFDLSVKAQYKKNKH

SEQ ID NO: 75 - protein, 50 aa, Artificial Sequence
  Artificial Sequence
  MISC_FEATURE (1)..(50): 36th amino acid(Xaa) is a 6-aminohexanoic acid. 37th amino acid(Xaa) is a D-form alanine. 39th amino acid(Xaa) is L-cyclohexylalanins. 49th amino acid(Xaa) is a D-form alanine. 50th amino acid(Xaa) is a 6-aminohexanoic acid.
GSHHHHHHGSDDDDKKTTKQSFDLSVKAQYKKNKHXXKXVAAWTLKAAXX

SEQ ID NO: 76 - protein, 50 aa, Artificial Sequence
  Artificial Sequence
  MISC_FEATURE (1)..(50): 21st amino acid(Xaa) is a 6-aminohexanoic acid. 22nd amino acid(Xaa) is a D-form alanine. 24th amino acid(Xaa) is L-cyclohexylalanins. 34th amino acid(Xaa) is a D-form alanine. 35th amino acid(Xaa) is a 6-aminohexanoic acid.
KTTKQSFDLSVKAQYKKNKHXXKXVAAWTLKAAXXGSHHHHHHGSDDDDK

SEQ ID NO: 77 - protein, 50 aa, Artificial Sequence
  Artificial Sequence
  MISC_FEATURE (1)..(50): 36th amino acid(Xaa) is a 6-aminohexanoic acid. 37th amino acid(Xaa) is a D-form alanine. 39th amino acid(Xaa) is L-cyclohexylalanins. 49th amino acid(Xaa) is a D-form alanine. 50th amino acid(Xaa) is a 6-aminohexanoic acid.
MRGSHHHHHHGSDDDDKIVDRNVPPIFNDVYWIAFXXKXVAAWTLKAAXX

SEQ ID NO: 78 - protein, 65 aa, Artificial Sequence
  Artificial Sequence
  MISC_FEATURE (1)..(65): 51st amino acid(Xaa) is a 6-aminohexanoic acid. 52nd amino acid(Xaa) is a D-form alanine. 54th amino acid(Xaa) is L-cyclohexylalanins. 64th amino acid(Xaa) is a D-form alanine. 65th amino acid(Xaa) is a 6-aminohexanoic acid.
MRGSHHHHHHGSDDDDKIVDGSHHHHHHGSDDDDKRNVPPIFNDVYWIAFXXKXVAAWTLKAAXX

SEQ ID NO: 79 - protein, 65 aa, Artificial Sequence
  Artificial Sequence
  MISC_FEATURE (1)..(65): 36th amino acid(Xaa) is a 6-aminohexanoic acid. 37th amino acid(Xaa) is a D-form alanine. 39th amino acid(Xaa) is L-cyclohexylalanins. 49th amino acid(Xaa) is a D-form alanine. 50th amino acid(Xaa) is a 6-aminohexanoic acid.
MRGSHHHHHHGSDDDDKIVDRNVPPIFNDVYWIAFXXKXVAAWTLKAAXXGSHHHHHHGSDDDDK

SEQ ID NO: 80 - protein, 30 aa, Artificial Sequence
  Artificial Sequence
RNVPPIFNDVYWIAFILMQYIKANSKFIGI

SEQ ID NO: 81 - protein, 47 aa, Artificial Sequence
  Artificial Sequence
RNVPPIFNDVYWIAFILMQYIKANSKFIGIPMGLPQSIALSSLMVAQ

SEQ ID NO: 82 - protein, 32 aa, Artificial Sequence
  Artificial Sequence
  MISC_FEATURE (1)..(32): 17th amino acid(Xaa) is a 6-aminohexanoic acid. 18th amino acid(Xaa) is a D-form alanine. 20th amino acid(Xaa) is L-cyclohexylalanins. 30th amino acid(Xaa) is a D-form alanine. 31st amino acid(Xaa) is a 6-aminohexanoic acid.
CRNVPPIFNDVYWIAFXXKXVAAWTLKAAXXC

SEQ ID NO: 83 - protein, 45 aa, Artificial Sequence
  Artificial Sequence
  MISC_FEATURE (1)..(45): 31st amino acid(Xaa) is a 6-aminohexanoic acid. 32nd amino acid(Xaa) is a D-form alanine. 34th amino acid(Xaa) is L-cyclohexylalanins. 44th amino acid(Xaa) is a D-form alanine. 45th amino acid(Xaa) is a 6-aminohexanoic acid.
RNVPPIFNDVYWIAFRNVPPIFNDVYWIAFXXKXVAAWTLKAAXX

SEQ ID NO: 84 - protein, 45 aa, Artificial Sequence
  Artificial Sequence
  MISC_FEATURE (1)..(45): 31st amino acid(Xaa) is a 6-aminohexanoic acid. 32nd amino acid(Xaa) is a D-form alanine. 34th amino acid(Xaa) is L-cyclohexylalanins. 44th amino acid(Xaa) is a D-form alanine. 45th amino acid(Xaa) is a 6-aminohexanoic acid.
RNVPPIFNDVYWIAFCRFRGLISLSQVYLSXXKXVAAWTLKAAXX

SEQ ID NO: 85 - protein, 50 aa, Artificial Sequence
  Artificial Sequence
  MISC_FEATURE (1)..(50): 36th amino acid(Xaa) is a 6-aminohexanoic acid. 37th amino acid(Xaa) is a D-form alanine. 39th amino acid(Xaa) is L-cyclohexylalanins. 49th amino acid(Xaa) is a D-form alanine. 50th amino acid(Xaa) is a 6-aminohexanoic acid.
RNVPPIFNDVYWIAFKTTKQSFDLSVKAQYKKNKHXXKXVAAWTLKAAXX

SEQ ID NO: 86 - protein, 45 aa, Artificial Sequence
  Artificial Sequence
  MISC_FEATURE (1)..(45): 31st amino acid(Xaa) is a 6-aminohexanoic acid. 32nd amino acid(Xaa) is a D-form alanine. 34th amino acid(Xaa) is L-cyclohexylalanins. 44th amino acid(Xaa) is a D-form alanine. 45th amino acid(Xaa) is a 6-aminohexanoic acid.
CRFRGLISLSQVYLSRNVPPIFNDVYWIAFXXKXVAAWTLKAAXX

SEQ ID NO: 87 - protein, 45 aa, Artificial Sequence
  Artificial Sequence
  MISC_FEATURE (1)..(45): 31st amino acid(Xaa) is a 6-aminohexanoic acid. 32nd amino acid(Xaa) is a D-form alanine. 34th amino acid(Xaa) is L-cyclohexylalanins. 44th amino acid(Xaa) is a D-form alanine. 45th amino acid(Xaa) is a 6-aminohexanoic acid.
CRFRGLISLSQVYLSCRFRGLISLSQVYLSXXKXVAAWTLKAAXX

SEQ ID NO: 88 - protein, 50 aa, Artificial Sequence
  Artificial Sequence
  MISC_FEATURE (1)..(50): 36th amino acid(Xaa) is a 6-aminohexanoic acid. 37th amino acid(Xaa) is a D-form alanine. 39th amino acid(Xaa) is L-cyclohexylalanins. 49th amino acid(Xaa) is a D-form alanine. 50th amino acid(Xaa) is a 6-aminohexanoic acid.
CRFRGLISLSQVYLSKTTKQSFDLSVKAQYKKNKHXXKXVAAWTLKAAXX

SEQ ID NO: 89 - protein, 50 aa, Artificial Sequence
  Artificial Sequence
  MISC_FEATURE (1)..(50): 36th amino acid(Xaa) is a 6-aminohexanoic acid. 37th amino acid(Xaa) is a D-form alanine. 39th amino acid(Xaa) is L-cyclohexylalanins. 49th amino acid(Xaa) is a D-form alanine. 50th amino acid(Xaa) is a 6-aminohexanoic acid.
KTTKQSFDLSVKAQYKKNKHRNVPPIFNDVYWIAFXXKXVAAWTLKAAXX

SEQ ID NO: 90 - protein, 50 aa, Artificial Sequence
  Artificial Sequence
  MISC_FEATURE (1)..(50): 36th amino acid(Xaa) is a 6-aminohexanoic acid. 37th amino acid(Xaa) is a D-form alanine. 39th amino acid(Xaa) is L-cyclohexylalanins. 49th amino acid(Xaa) is a D-form alanine. 50th amino acid(Xaa) is a 6-aminohexanoic acid.
KTTKQSFDLSVKAQYKKNKHCRFRGLISLSQVYLSXXKXVAAWTLKAAXX

SEQ ID NO: 91 - protein, 55 aa, Artificial Sequence
  Artificial Sequence
  MISC_FEATURE (1)..(55): 41st amino acid(Xaa) is a 6-aminohexanoic acid. 42nd amino acid(Xaa) is a D-form alanine. 44th amino acid(Xaa) is L-cyclohexylalanins. 54th amino acid(Xaa) is a D-form alanine. 55th amino acid(Xaa) is a 6-aminohexanoic acid.
KTTKQSFDLSVKAQYKKNKHKTTKQSFDLSVKAQYKKNKHXXKXVAAWTLKAAXX

SEQ ID NO: 92 - protein, 41 aa, Artificial Sequence
  Artificial Sequence
  MISC_FEATURE (1)..(41): 32nd amino acid(Xaa) is L-cyclohexylalanins.
RNVPPIFNDVYWIAFCRFRGLISLSQVYLSKXVAAWTLKAA

SEQ ID NO: 93 - protein, 33 aa, Artificial Sequence
  Artificial Sequence
  MISC_FEATURE (1)..(33): 24th amino acid(Xaa) is L-cyclohexylalanins.
PIFNDVYWIAFGLISLSQVYLSKXVAAWTLKAA

SEQ ID NO: 94 - protein, 33 aa, Artificial Sequence
  Artificial Sequence
  MISC_FEATURE (1)..(33): 24th amino acid(Xaa) is L-cyclohexylalanins.
RNVPPIFNDVYCRFRGLISLSQKXVAAWTLKAA

SEQ ID NO: 95 - protein, 33 aa, Artificial Sequence
  Artificial Sequence
  MISC_FEATURE (1)..(33): 24th amino acid(Xaa) is L-cyclohexylalanins.
PIFNDVYWIAFCRFRGLISLSQKXVAAWTLKAA

SEQ ID NO: 96 - protein, 29 aa, Artificial Sequence
  Artificial Sequence
  MISC_FEATURE (1)..(29): 20th amino acid(Xaa) is L-cyclohexylalanins.
PPIFNDVYWRGLISLSQVKXVAAWTLKAA

SEQ ID NO: 97 - protein, 47 aa, Artificial Sequence
  Artificial Sequence
  MISC_FEATURE (1)..(47): 32nd amino acid(Xaa) is L-cyclohexylalanins.
RNVPPIFNDVYWIAFCRFRGLISLSQVYLSKXVAAWTLKAAHHHHHH

SEQ ID NO: 98 - protein, 65 aa, Artificial Sequence
  Artificial Sequence
  MISC_FEATURE (1)..(65): 51st amino acid(Xaa) is a 6-aminohexanoic acid. 52nd amino acid(Xaa) is a D-form alanine. 54th amino acid(Xaa) is L-cyclohexylalanins. 64th amino acid(Xaa) is a D-form alanine. 65th amino acid(Xaa) is a 6-aminohexanoic acid.
MRGSHHHHHHGSDDDDKIVDRNVPPIFNDVYWIAFCRFRGLISLSQVYLSXXKXVAAWTLKAAXX

SEQ ID NO: 99 - protein, 63 aa, Artificial Sequence
  Artificial Sequence
  MISC_FEATURE (1)..(63): 51st amino acid(Xaa) is a 6-aminohexanoic acid. 52nd amino acid(Xaa) is a D-form alanine. 54th amino acid(Xaa) is L-cyclohexylalanins. 64th amino acid(Xaa) is a D-form alanine. 65th amino acid(Xaa) is a 6-aminohexanoic acid.
MRGSHHHHHHGSDDDDKIVDRNVPPIFNDVYWIAFCRFRGLISLSQVYLSXXKXVAAWTLKAA

SEQ ID NO: 100 - protein, 43 aa, Artificial Sequence
  Artificial Sequence
  MISC_FEATURE (1)..(43): 31st amino acid(Xaa) is a 6-aminohexanoic acid. 32nd amino acid(Xaa) is a D-form alanine. 34th amino acid(Xaa) is L-cyclohexylalanins. 44th amino acid(Xaa) is a D-form alanine. 45th amino acid(Xaa) is a 6-aminohexanoic acid.
RNVPPIFNDVYWIAFCRFRGLISLSQVYLSXXKXVAAWTLKAA

SEQ ID NO: 101 - protein, 76 aa, Artificial Sequence
  Artificial Sequence
  MISC_FEATURE (1)..(76): 64th amino acid(Xaa) is a 6-aminohexanoic acid. 65th amino acid(Xaa) is a D-form alanine. 67th amino acid(Xaa) is L-cyclohexylalanins. 77th amino acid(Xaa) is a D-form alanine. 78th amino acid(Xaa) is a 6-aminohexanoic acid.
MRGSHHHHHHGSDDDDKIVDRNVPPIFNDVYWIAFGGGGSGGGGGGSSRNVPPIFNDVYWIAFXXKXVAAWTLKAA

SEQ ID NO: 102 - protein, 56 aa, Artificial Sequence
  Artificial Sequence
  MISC_FEATURE (1)..(56): 44th amino acid(Xaa) is a 6-aminohexanoic acid. 45th amino acid(Xaa) is a D-form alanine. 47th amino acid(Xaa) is L-cyclohexylalanins. 57th amino acid(Xaa) is a D-form alanine. 58th amino acid(Xaa) is a 6-aminohexanoic acid.
RNVPPIFNDVYWIAFGGGGSGGGGGGSSRNVPPIFNDVYWIAFXXKXVAAWTLKAA

SEQ ID NO: 103 - protein, 58 aa, Artificial Sequence
  Artificial Sequence
  MISC_FEATURE (1)..(58): 44th amino acid(Xaa) is a 6-aminohexanoic acid. 45th amino acid(Xaa) is a D-form alanine. 47th amino acid(Xaa) is L-cyclohexylalanins. 57th amino acid(Xaa) is a D-form alanine. 58th amino acid(Xaa) is a 6-aminohexanoic acid.
RNVPPIFNDVYWIAFGGGGSGGGGGGSSRNVPPIFNDVYWIAFXXKXVAAWTLKAAXX

SEQ ID NO: 104 - protein, 45 aa, Artificial Sequence
  Artificial Sequence
RNVPPIFNDVYWIAFRNVPPIFNDVYWIAFILMQYIKANSKFIGI

SEQ ID NO: 105 - protein, 62 aa, Artificial Sequence
  Artificial Sequence
RNVPPIFNDVYWIAFRNVPPIFNDVYWIAFILMQYIKANSKFIGIPMGLPQSIALSSLMVAQ

SEQ ID NO: 106 - protein, 47 aa, Artificial Sequence
  Artificial Sequence
  MISC_FEATURE (1)..(47): 32nd amino acid(Xaa) is a 6-aminohexanoic acid. 33rd amino acid(Xaa) is a D-form alanine. 35th amino acid(Xaa) is L-cyclohexylalanins. 45th amino acid(Xaa) is a D-form alanine. 46th amino acid(Xaa) is a 6-aminohexanoic acid.
CRNVPPIFNDVYWIAFCRFRGLISLSQVYLSXXKXVAAWTLKAAXXC

SEQ ID NO: 107 - protein, 45 aa, Artificial Sequence
  Artificial Sequence
  MISC_FEATURE (1)..(45): 16th amino acid(Xaa) is a 6-aminohexanoic acid. 17th amino acid(Xaa) is a D-form alanine. 19th amino acid(Xaa) is L-cyclohexylalanins. 29th amino acid(Xaa) is a D-form alanine. 30th amino acid(Xaa) is a 6-aminohexanoic acid.
RNVPPIFNDVYWIAFXXKXVAAWTLKAAXXRNVPPIFNDVYWIAF

SEQ ID NO: 108 - protein, 45 aa, Artificial Sequence
  Artificial Sequence
  MISC_FEATURE (1)..(45): 16th amino acid(Xaa) is a 6-aminohexanoic acid. 17th amino acid(Xaa) is a D-form alanine. 19th amino acid(Xaa) is L-cyclohexylalanins. 29th amino acid(Xaa) is a D-form alanine. 30th amino acid(Xaa) is a 6-aminohexanoic acid.
RNVPPIFNDVYWIAFXXKXVAAWTLKAAXXCRFRGLISLSQVYLS

SEQ ID NO: 109 - protein, 50 aa, Artificial Sequence
  Artificial Sequence
  MISC_FEATURE (1)..(50): 16th amino acid(Xaa) is a 6-aminohexanoic acid. 17th amino acid(Xaa) is a D-form alanine. 19th amino acid(Xaa) is L-cyclohexylalanins. 29th amino acid(Xaa) is a D-form alanine. 30th amino acid(Xaa) is a 6-aminohexanoic acid.
RNVPPIFNDVYWIAFXXKXVAAWTLKAAXXKTTKQSFDLSVKAQYKKNKH

SEQ ID NO: 110 - protein, 45 aa, Artificial Sequence
  Artificial Sequence
  MISC_FEATURE (1)..(45): 16th amino acid(Xaa) is a 6-aminohexanoic acid. 17th amino acid(Xaa) is a D-form alanine. 19th amino acid(Xaa) is L-cyclohexylalanins. 29th amino acid(Xaa) is a D-form alanine. 30th amino acid(Xaa) is a 6-aminohexanoic acid.
CRFRGLISLSQVYLSXXKXVAAWTLKAAXXRNVPPIFNDVYWIAF

SEQ ID NO: 111 - protein, 45 aa, Artificial Sequence
  Artificial Sequence
  MISC_FEATURE (1)..(45): 16th amino acid(Xaa) is a 6-aminohexanoic acid. 17th amino acid(Xaa) is a D-form alanine. 19th amino acid(Xaa) is L-cyclohexylalanins. 29th amino acid(Xaa) is a D-form alanine. 30th amino acid(Xaa) is a 6-aminohexanoic acid.
CRFRGLISLSQVYLSXXKXVAAWTLKAAXXCRFRGLISLSQVYLS

SEQ ID NO: 112 - protein, 50 aa, Artificial Sequence; identical to SEQ ID NO: 109
  Artificial Sequence
  MISC_FEATURE (1)..(50): 16th amino acid(Xaa) is a 6-aminohexanoic acid. 17th amino acid(Xaa) is a D-form alanine. 19th amino acid(Xaa) is L-cyclohexylalanins. 29th amino acid(Xaa) is a D-form alanine. 30th amino acid(Xaa) is a 6-aminohexanoic acid.

SEQ ID NO: 113 - protein, 50 aa, Artificial Sequence
  Artificial Sequence
  MISC_FEATURE (1)..(50): 21st amino acid(Xaa) is a 6-aminohexanoic acid. 22nd amino acid(Xaa) is a D-form alanine. 24th amino acid(Xaa) is L-cyclohexylalanins. 34th amino acid(Xaa) is a D-form alanine. 35th amino acid(Xaa) is a 6-aminohexanoic acid.
KTTKQSFDLSVKAQYKKNKHXXKXVAAWTLKAAXXRNVPPIFNDVYWIAF

SEQ ID NO: 114 - protein, 50 aa, Artificial Sequence
  Artificial Sequence
  MISC_FEATURE (1)..(50): 21st amino acid(Xaa) is a 6-aminohexanoic acid. 22nd amino acid(Xaa) is a D-form alanine. 24th amino acid(Xaa) is L-cyclohexylalanins. 34th amino acid(Xaa) is a D-form alanine. 35th amino acid(Xaa) is a 6-aminohexanoic acid.
KTTKQSFDLSVKAQYKKNKHXXKXVAAWTLKAAXXCRFRGLISLSQVYLS

SEQ ID NO: 115 - protein, 55 aa, Artificial Sequence
  Artificial Sequence
  MISC_FEATURE (1)..(55): 21st amino acid(Xaa) is a 6-aminohexanoic acid. 22nd amino acid(Xaa) is a D-form alanine. 24th amino acid(Xaa) is L-cyclohexylalanins. 34th amino acid(Xaa) is a D-form alanine. 35th amino acid(Xaa) is a 6-aminohexanoic acid.
KTTKQSFDLSVKAQYKKNKHXXKXVAAWTLKAAXXKTTKQSFDLSVKAQYKKNKH

SEQ ID NO: 116 - protein, 33 aa, Artificial Sequence
  Artificial Sequence
  MISC_FEATURE (1)..(33): 13rd amino acid(Xaa) is L-cyclohexylalanins.
PIFNDVYWIAFKXVAAWTLKAACRFRGLISLSQ

SEQ ID NO: 117 - protein, 29 aa, Artificial Sequence
  Artificial Sequence
PPIFNDVYWKXVAAWTLKAARGLISLSQV

SEQ ID NO: 118 - protein, 65 aa, Artificial Sequence
  Artificial Sequence
  MISC_FEATURE (1)..(65): 36th amino acid(Xaa) is a 6-aminohexanoic acid. 37th amino acid(Xaa) is a D-form alanine. 39th amino acid(Xaa) is L-cyclohexylalanins. 49th amino acid(Xaa) is a D-form alanine. 50th amino acid(Xaa) is a 6-aminohexanoic acid.
MRGSHHHHHHGSDDDDKIVDRNVPPIFNDVYWIAFXXKXVAAWTLKAAXXRNVPPIFNDVYWIAF

SEQ ID NO: 119 - protein, 108 aa, Artificial Sequence
  Artificial Sequence
MRGSHHHHHHGSDDDDKIVDRNVPPIFNDVYWIAFGGGGSGGGGGGSSILMQYIKANSKFIGIPMGLPQSIALSSLMVAQGGGGSGGGGGGSSCRFRGLISLSQVYLS

SEQ ID NO: 120 - protein, 45 aa, Artificial Sequence
  Artificial Sequence
RNVPPIFNDVYWIAFILMQYIKANSKFIGICRFRGLISLSQVYLS

SEQ ID NO: 121 - protein, 45 aa, Artificial Sequence
  Artificial Sequence
  MISC_FEATURE (1)..(45): 16th amino acid(Xaa) is a 6-aminohexanoic acid. 17th amino acid(Xaa) is a D-form alanine. 19th amino acid(Xaa) is L-cyclohexylalanins. 29th amino acid(Xaa) is a D-form alanine. 30th amino acid(Xaa) is a 6-aminohexanoic acid.
RNVPPIFNDVYWIAFXPKYVKQNTLKLATXCRFRGLISLSQVYLS

SEQ ID NO: 122 - protein, 47 aa, Artificial Sequence
  Artificial Sequence
  MISC_FEATURE (1)..(47): 17th amino acid(Xaa) is a 6-aminohexanoic acid. 18th amino acid(Xaa) is a D-form alanine. 20th amino acid(Xaa) is L-cyclohexylalanins. 30th amino acid(Xaa) is a D-form alanine. 31st amino acid(Xaa) is a 6-aminohexanoic acid.
CRNVPPIFNDVYWIAFXXKXVAAWTLKAAXXRNVPPIFNDVYWIAFC

SEQ ID NO: 123 - protein, 45 aa, Artificial Sequence
  Artificial Sequence
  MISC_FEATURE (1)..(45): 16th amino acid(Xaa) is a 6-aminohexanoic acid. 17th amino acid(Xaa) is a D-form alanine. 19th amino acid(Xaa) is L-cyclohexylalanins. 29th amino acid(Xaa) is a D-form alanine. 30th amino acid(Xaa) is a 6-aminohexanoic acid.
RNVPPIFNDVYWIAFXXKXVAAWTLKAAXXILMQYIKANSKFIGI

SEQ ID NO: 124 - protein, 45 aa, Artificial Sequence
  Artificial Sequence
  MISC_FEATURE (1)..(45): 16th amino acid(Xaa) is a 6-aminohexanoic acid. 17th amino acid(Xaa) is a D-form alanine. 19th amino acid(Xaa) is L-cyclohexylalanins. 29th amino acid(Xaa) is a D-form alanine. 30th amino acid(Xaa) is a 6-aminohexanoic acid.
CRFRGLISLSQVYLSXXKXVAAWTLKAAXXILMQYIKANSKFIGI

SEQ ID NO: 125 - protein, 50 aa, Artificial Sequence
  Artificial Sequence
  MISC_FEATURE (1)..(50): 21st amino acid(Xaa) is a 6-aminohexanoic acid. 22nd amino acid(Xaa) is a D-form alanine. 24th amino acid(Xaa) is L-cyclohexylalanins. 34th amino acid(Xaa) is a D-form alanine. 35th amino acid(Xaa) is a 6-aminohexanoic acid.
KTTKQSFDLSVKAQYKKNKHXXKXVAAWTLKAAXXILMQYIKANSKFIGI

SEQ ID NO: 126 - protein, 45 aa, Artificial Sequence
  Artificial Sequence
  MISC_FEATURE (1)..(45): 16th amino acid(Xaa) is a 6-aminohexanoic acid. 17th amino acid(Xaa) is a D-form alanine. 19th amino acid(Xaa) is L-cyclohexylalanins. 29th amino acid(Xaa) is a D-form alanine. 30th amino acid(Xaa) is a 6-aminohexanoic acid.
ILMQYIKANSKFIGIXXKXVAAWTLKAAXXRNVPPIFNDVYWIAF

SEQ ID NO: 127 - protein, 45 aa, Artificial Sequence
  Artificial Sequence
  MISC_FEATURE (1)..(45): 16th amino acid(Xaa) is a 6-aminohexanoic acid. 17th amino acid(Xaa) is a D-form alanine. 19th amino acid(Xaa) is L-cyclohexylalanins. 29th amino acid(Xaa) is a D-form alanine. 30th amino acid(Xaa) is a 6-aminohexanoic acid.
ILMQYIKANSKFIGIXXKXVAAWTLKAAXXCRFRGLISLSQVYLS

SEQ ID NO: 128 - protein, 50 aa, Artificial Sequence
  Artificial Sequence
  MISC_FEATURE (1)..(50): 16th amino acid(Xaa) is a 6-aminohexanoic acid. 17th amino acid(Xaa) is a D-form alanine. 19th amino acid(Xaa) is L-cyclohexylalanins. 29th amino acid(Xaa) is a D-form alanine. 30th amino acid(Xaa) is a 6-aminohexanoic acid.
ILMQYIKANSKFIGIXXKXVAAWTLKAAXXKTTKQSFDLSVKAQYKKNKH

SEQ ID NO: 129 - protein, 33 aa, Artificial Sequence
  Artificial Sequence
  MISC_FEATURE (1)..(33): 13rd amino acid(Xaa) is L-cyclohexylalanins. 24th amino acid(Xaa) is L-cyclohexylalanins.
PIFNDVYWIAFKXVAAWTLKAAKXVAAWTLKAA

SEQ ID NO: 130 - protein, 31 aa, Artificial Sequence
  Artificial Sequence
  MISC_FEATURE (1)..(31): 11st amino acid(Xaa) is L-cyclohexylalanins. 21st amino acid(Xaa) is L-cyclohexylalanins.
PPIFNDVYWKXVAAWTLKAAKXVAAWTLKAA

SEQ ID NO: 131 - protein, 65 aa, Artificial Sequence
  Artificial Sequence
  MISC_FEATURE (1)..(65): 36th amino acid(Xaa) is a 6-aminohexanoic acid. 37th amino acid(Xaa) is a D-form alanine. 39th amino acid(Xaa) is L-cyclohexylalanins. 49th amino acid(Xaa) is a D-form alanine. 50th amino acid(Xaa) is a 6-aminohexanoic acid.
MRGSHHHHHHGSDDDDKIVDRNVPPIFNDVYWIAFXXKXVAAWTLKAAXXILMQYIKANSKFIGI

SEQ ID NO: 132 - protein, 50 aa, Artificial Sequence
  Artificial Sequence
  MISC_FEATURE (1)..(50): 36th amino acid(Xaa) is a 6-aminohexanoic acid. 37th amino acid(Xaa) is a D-form alanine. 39th amino acid(Xaa) is L-cyclohexylalanins. 49th amino acid(Xaa) is a D-form alanine. 50th amino acid(Xaa) is a 6-aminohexanoic acid.
MRGSHHHHHHGSDDDDKIVDILMQYIKANSKFIGIXXKXVAAWTLKAAXX

SEQ ID NO: 133 - protein, 78 aa, Artificial Sequence
  Artificial Sequence
  MISC_FEATURE (1)..(78): 49th amino acid(Xaa) is a 6-aminohexanoic acid. 50th amino acid(Xaa) is a D-form alanine. 52nd amino acid(Xaa) is L-cyclohexylalanins. 62nd amino acid(Xaa) is a D-form alanine. 63rd amino acid(Xaa) is a 6-aminohexanoic acid.
MRGSHHHHHHGSDDDDKIVDRNVPPIFNDVYWIAFGGGGSGGGGGGSSXXKXVAAWTLKAAXXILMQYIKANSKFIGI

SEQ ID NO: 134 - protein, 125 aa, Artificial Sequence
  Artificial Sequence
MRGSHHHHHHGSDDDDKIVDRNVPPIFNDVYWIAFGGGGSGGGGGGSSILMQYIKANSKFIGIPMGLPQSIALSSLMVAQGGGGSGGGGGGSSILMQYIKANSKFIGIPMGLPQSIALSSLMVAQ

SEQ ID NO: 135 - protein, 43 aa, Artificial Sequence
  Artificial Sequence
  MISC_FEATURE (1)..(43): 16th amino acid(Xaa) is a 6-aminohexanoic acid. 17th amino acid(Xaa) is a D-form alanine. 19th amino acid(Xaa) is L-cyclohexylalanins. 29th amino acid(Xaa) is a D-form alanine. 30th amino acid(Xaa) is a 6-aminohexanoic acid. 32nd amino acid(Xaa) is L-cyclohex
RNVPPIFNDVYWIAFXXKXVAAWTLKAAXXKXLAAFTIRAAXX

SEQ ID NO: 136 - protein, 47 aa, Artificial Sequence
  Artificial Sequence
  MISC_FEATURE (1)..(47): 17th amino acid(Xaa) is a 6-aminohexanoic acid. 18th amino acid(Xaa) is a D-form alanine. 20th amino acid(Xaa) is L-cyclohexylalanins. 30th amino acid(Xaa) is a D-form alanine. 31st amino acid(Xaa) is a 6-aminohexanoic acid.
CRNVPPIFNDVYWIAFXXKXVAAWTLKAAXXILMQYIKANSKFIGIC

SEQ ID NO: 137 - protein, 60 aa, Artificial Sequence
  Artificial Sequence
  MISC_FEATURE (1)..(60): 16th amino acid(Xaa) is a 6-aminohexanoic acid. 17th amino acid(Xaa) is a D-form alanine. 19th amino acid(Xaa) is L-cyclohexylalanins. 29th amino acid(Xaa) is a D-form alanine. 30th amino acid(Xaa) is a 6-aminohexanoic acid.
RNVPPIFNDVYWIAFXXKXVAAWTLKAAXXILMQYIKANSKFIGIRNVPPIFNDVYWIAF

SEQ ID NO: 138 - protein, 60 aa, Artificial Sequence
  Artificial Sequence
  MISC_FEATURE (1)..(60): 16th amino acid(Xaa) is a 6-aminohexanoic acid. 17th amino acid(Xaa) is a D-form alanine. 19th amino acid(Xaa) is L-cyclohexylalanins. 29th amino acid(Xaa) is a D-form alanine. 30th amino acid(Xaa) is a 6-aminohexanoic acid.
RNVPPIFNDVYWIAFXXKXVAAWTLKAAXXILMQYIKANSKFIGICRFRGLISLSQVYLS

SEQ ID NO: 139 - protein, 65 aa, Artificial Sequence
  Artificial Sequence
  MISC_FEATURE (1)..(65): 16th amino acid(Xaa) is a 6-aminohexanoic acid. 17th amino acid(Xaa) is a D-form alanine. 19th amino acid(Xaa) is L-cyclohexylalanins. 29th amino acid(Xaa) is a D-form alanine. 30th amino acid(Xaa) is a 6-aminohexanoic acid.
RNVPPIFNDVYWIAFXXKXVAAWTLKAAXXILMQYIKANSKFIGIKTTKQSFDLSVKAQYKKNKH

SEQ ID NO: 140 - protein, 60 aa, Artificial Sequence
  Artificial Sequence
  MISC_FEATURE (1)..(60): 16th amino acid(Xaa) is a 6-aminohexanoic acid. 17th amino acid(Xaa) is a D-form alanine. 19th amino acid(Xaa) is L-cyclohexylalanins. 29th amino acid(Xaa) is a D-form alanine. 30th amino acid(Xaa) is a 6-aminohexanoic acid.
CRFRGLISLSQVYLSXXKXVAAWTLKAAXXILMQYIKANSKFIGIRNVPPIFNDVYWIAF

SEQ ID NO: 141 - protein, 60 aa, Artificial Sequence
  Artificial Sequence
  MISC_FEATURE (1)..(60): 16th amino acid(Xaa) is a 6-aminohexanoic acid. 17th amino acid(Xaa) is a D-form alanine. 19th amino acid(Xaa) is L-cyclohexylalanins. 29th amino acid(Xaa) is a D-form alanine. 30th amino acid(Xaa) is a 6-aminohexanoic acid.
CRFRGLISLSQVYLSXXKXVAAWTLKAAXXILMQYIKANSKFIGICRFRGLISLSQVYLS

SEQ ID NO: 142 - protein, 65 aa, Artificial Sequence
  Artificial Sequence
  MISC_FEATURE (1)..(65): 16th amino acid(Xaa) is a 6-aminohexanoic acid. 17th amino acid(Xaa) is a D-form alanine. 19th amino acid(Xaa) is L-cyclohexylalanins. 29th amino acid(Xaa) is a D-form alanine. 30th amino acid(Xaa) is a 6-aminohexanoic acid.
CRFRGLISLSQVYLSXXKXVAAWTLKAAXXILMQYIKANSKFIGIKTTKQSFDLSVKAQYKKNKH

SEQ ID NO: 143 - protein, 65 aa, Artificial Sequence
  Artificial Sequence
  MISC_FEATURE (1)..(65): 21st amino acid(Xaa) is a 6-aminohexanoic acid. 22nd amino acid(Xaa) is a D-form alanine. 24th amino acid(Xaa) is L-cyclohexylalanins. 34th amino acid(Xaa) is a D-form alanine. 35th amino acid(Xaa) is a 6-aminohexanoic acid.
KTTKQSFDLSVKAQYKKNKHXXKXVAAWTLKAAXXILMQYIKANSKFIGIRNVPPIFNDVYWIAF

SEQ ID NO: 144 - protein, 65 aa, Artificial Sequence
  Artificial Sequence
  MISC_FEATURE (1)..(65): 21st amino acid(Xaa) is a 6-aminohexanoic acid. 22nd amino acid(Xaa) is a D-form alanine. 24th amino acid(Xaa) is L-cyclohexylalanins. 34th amino acid(Xaa) is a D-form alanine. 35th amino acid(Xaa) is a 6-aminohexanoic acid.
KTTKQSFDLSVKAQYKKNKHXXKXVAAWTLKAAXXILMQYIKANSKFIGICRFRGLISLSQVYLS

SEQ ID NO: 145 - protein, 70 aa, Artificial Sequence
  Artificial Sequence
  MISC_FEATURE (1)..(70): 21st amino acid(Xaa) is a 6-aminohexanoic acid. 22nd amino acid(Xaa) is a D-form alanine. 24th amino acid(Xaa) is L-cyclohexylalanins. 34th amino acid(Xaa) is a D-form alanine. 35th amino acid(Xaa) is a 6-aminohexanoic acid.
KTTKQSFDLSVKAQYKKNKHXXKXVAAWTLKAAXXILMQYIKANSKFIGIKTTKQSFDLSVKAQYKKNKH

SEQ ID NO: 146 - protein, 80 aa, Artificial Sequence
  Artificial Sequence
  MISC_FEATURE (1)..(80): 36th amino acid(Xaa) is a 6-aminohexanoic acid. 37th amino acid(Xaa) is a D-form alanine. 39th amino acid(Xaa) is L-cyclohexylalanins. 49th amino acid(Xaa) is a D-form alanine. 50th amino acid(Xaa) is a 6-aminohexanoic acid.
MRGSHHHHHHGSDDDDKIVDRNVPPIFNDVYWIAFXXKXVAAWTLKAAXXILMQYIKANSKFIGIRNVPPIFNDVYWIAF

SEQ ID NO: 147 - protein, 140 aa, Artificial Sequence
  Artificial Sequence
MRGSHHHHHHGSDDDDKIVDRNVPPIFNDVYWIAFGGGGSGGGGGGSSILMQYIKANSKFIGIPMGLPQSIALSSLMVAQILMQYIKANSKFIGIPMGLPQSIALSSLMVAQGGGGSGGGGGGSSCRFRGLISLSQVYLS

SEQ ID NO: 148 - protein, 44 aa, Artificial Sequence
  Artificial Sequence
  MISC_FEATURE (1)..(44): 13rd amino acid(Xaa) is L-cyclohexylalanins. 24th amino acid(Xaa) is L-cyclohexylalanins.
PIFNDVYWIAFKXVAAWTLKAAKXVAAWTLKAACRFRGLISLSQ

SEQ ID NO: 149 - protein, 40 aa, Artificial Sequence
  Artificial Sequence
  MISC_FEATURE (1)..(40): 11st amino acid(Xaa) is L-cyclohexylalanins. 22nd amino acid(Xaa) is L-cyclohexylalanins.
PPIFNDVYWKXVAAWTLKAAKXVAAWTLKAARGLISLSQV

SEQ ID NO: 150 - protein, 62 aa, Artificial Sequence
  Artificial Sequence
  MISC_FEATURE (1)..(62): 17th amino acid(Xaa) is a 6-aminohexanoic acid. 18th amino acid(Xaa) is a D-form alanine. 20th amino acid(Xaa) is L-cyclohexylalanins. 30th amino acid(Xaa) is a D-form alanine. 31st amino acid(Xaa) is a 6-aminohexanoic acid.
CRNVPPIFNDVYWIAFXXKXVAAWTLKAAXXILMQYIKANSKFIGIRNVPPIFNDVYWIAFC

SEQ ID NO: 151 - protein, 80 aa, Artificial Sequence
  Artificial Sequence
  MISC_FEATURE (1)..(80): Each of 36th, 50th, 66th, and 80th amino acid(Xaa) is a 6-aminohexanoic acid. Each of 37th, 49th, 67th, and 79th amino acid(Xaa) is a D-form alanine. Each of 39th and 69th amino acid(Xaa) is L-cyclohexylalanins.
MRGSHHHHHHGSDDDDKIVDRNVPPIFNDVYWIAFXXKXVAAWTLKAAXXRNVPPIFNDVYWIAFXXKXVAAWTLKAAXX

SEQ ID NO: 152 - protein, 90 aa, Artificial Sequence
  Artificial Sequence
  MISC_FEATURE (1)..(90): Each of 31st, 45th, 76th, and 90th amino acid(Xaa) is a 6-aminohexanoic acid. Each of 32nd, 44th, 77th, and 89th amino acid(Xaa) is a D-form alanine. Each of 34th and 79th amino acid(Xaa) is L-cyclohexylalanins.
RNVPPIFNDVYWIAFCRFRGLISLSQVYLSXXKXVAAWTLKAAXXRNVPPIFNDVYWIAFCRFRGLISLSQVYLSXXKXVAAWTLKAAXX

SEQ ID NO: 153 - protein, 90 aa, Artificial Sequence
  Artificial Sequence
  MISC_FEATURE (1)..(90): Each of 16th, 30th, 61st, and 75th amino acid(Xaa) is a 6-aminohexanoic acid. Each of 17th, 29th, 62nd, and 74th amino acid(Xaa) is a D-form alanine. Each of 19th and 64th amino acid(Xaa) is L-cyclohexylalanins.
RNVPPIFNDVYWIAFXXKXVAAWTLKAAXXCRFRGLISLSQVYLSRNVPPIFNDVYWIAFXXKXVAAWTLKAAXXCRFRGLISLSQVYLS

SEQ ID NO: 154 - protein, 90 aa, Artificial Sequence
  Artificial Sequence
  MISC_FEATURE (1)..(90): Each of 16th, 30th, 61st, and 75th amino acid(Xaa) is a 6-aminohexanoic acid. Each of 17th, 29th, 62nd and 74th amino acid(Xaa) is a D-form alanine. Each of 19th and 64th amino acid(Xaa) is L-cyclohexylalanins.
RNVPPIFNDVYWIAFXXKXVAAWTLKAAXXILMQYIKANSKFIGIRNVPPIFNDVYWIAFXXKXVAAWTLKAAXXILMQYIKANSKFIGI

SEQ ID NO: 155 - protein, 120 aa, Artificial Sequence
  Artificial Sequence
  MISC_FEATURE (1)..(120): Each of 16th, 30th, 76th, and 90th amino acid(Xaa) is a 6-aminohexanoic acid. Each of 17th, 29th, 77th, and 89th amino acid(Xaa) is a D-form alanine. Each of 19th and 79th amino acid(Xaa) is L-cyclohexylalanins.
RNVPPIFNDVYWIAFXXKXVAAWTLKAAXXILMQYIKANSKFIGIRNVPPIFNDVYWIAFRNVPPIFNDVYWIAFXXKXVAAWTLKAAXXILMQYIKANSKFIGIRNVPPIFNDVYWIAF

SEQ ID NO: 156 - protein, 75 aa, Artificial Sequence
  Artificial Sequence
  MISC_FEATURE (1)..(75): Each of 16th, 30th, 61st, and 75th amino acid(Xaa) is a 6-aminohexanoic acid. Each of 17th, 29th, 62nd, and 74th amino acid(Xaa) is a D-form alanine. Each of 19th and 64th amino acid(Xaa) is L-cyclohexylalanins.
RNVPPIFNDVYWIAFXXKXVAAWTLKAAXXRNVPPIFNDVYWIAFCRFRGLISLSQVYLSXXKXVAAWTLKAAXX

SEQ ID NO: 157 - protein, 30 aa, Artificial Sequence
  Artificial Sequence
  MISC_FEATURE (1)..(30): Each of 16th, 30th, 46th, 62nd, 76th, 92nd, 108th, and 122nd amino acid(Xaa) is a 6-aminohexanoic acid. Each of 17th, 29th, 63rd, 75th, 109th, and 121st amino acid(Xaa) is a D-form alanine. Each of 19th, 65th, and 111st amino acid(Xaa) is L-cyclohexylalanins.
ILMQYIKANSKFIGICRFRGLISLSQVYLS

SEQ ID NO: 158 - protein, 272 aa, Artificial Sequence
  Artificial Sequence
  MISC_FEATURE (1)..(272): Each of 16th, 30th, 61st, 75th, 106th, 120th, 136th, 150th, 166th, 182nd, 196th, 212nd, 228th, and 242nd amino acid(Xaa) is a 6-aminohexanoic acid. Each of 17th, 29th, 62nd, 74th, 107th, 119th, 137th, 149th, 183rd, 195th, 229th, and 241st amino acid(Xaa) is a
RNVPPIFNDVYWIAFXXKXVAAWTLKAAXXRNVPPIFNDVYWIAFCRFRGLISLSQVYLSXXKXVAAWTLKAAXXRNVPPIFNDVYWIAFCRFRGLISLSQVYLSXXKXVAAWTLKAAXXRNVPPIFNDVYWIAFXXKXVAAWTLKAAXXRNVPPIFNDVYWIAFXRNVPPIFNDVYWIAFXXKXVAAWTLKAAXXILMQYIKANSKFIGIXRNVPPIFNDVYWIAFXXKXVAAWTLKAAXXILMQYIKANSKFIGICRFRGLISLSQVYLS

SEQ ID NO: 159 - protein, 6 aa, Artificial Sequence
  Artificial Sequence
RRRRRR

SEQ ID NO: 160 - protein, 43 aa, Artificial Sequence
  Unit peptide
  MISC_FEATURE (1)..(43): Xaa at position 19 is L-cyclohexylalanine
RNVPPIFNDVYWIAFXXKXVAAWTLKAACRFRGLISLSQVYLS

SEQ ID NO: 161 - protein, 30 aa, Artificial Sequence
  Unit peptide
  MISC_FEATURE (1)..(30): Xaa at position 19 is L-cyclohexylalanine
RNVPPIFNDVYWIAFXXKXVAAWTLKAACR

SEQ ID NO: 162 - protein, 10 aa, Artificial Sequence
  Th epitope
PLGFFPDHQL

SEQ ID NO: 163 - protein, 16 aa, Artificial Sequence
  Th epitope
WPEANQVGAGAFGPGF

SEQ ID NO: 164 - protein, 15 aa, Artificial Sequence
  Th epitope
MQWNSTALHQALQDP

SEQ ID NO: 165 - protein, 26 aa, Artificial Sequence
  Th epitope
MQWNSTTFHQTLQDPRVRGLYFPAGG

SEQ ID NO: 166 - protein, 10 aa, Artificial Sequence
  Th epitope
FFLLTRILTI

SEQ ID NO: 167 - protein, 15 aa, Artificial Sequence
  Th epitope
FFLLTRILTIPQSLD

SEQ ID NO: 168 - protein, 15 aa, Artificial Sequence
  Th epitope
TSLNFLGGTTVCLGQ

SEQ ID NO: 169 - protein, 16 aa, Artificial Sequence
  Th epitope
QSPTSNHSPTSCPPIC

SEQ ID NO: 170 - protein, 19 aa, Artificial Sequence
  Th epitope
IIFLFILLLCLIFLLVLLD

SEQ ID NO: 171 - protein, 14 aa, Artificial Sequence
  Th epitope
CTTPAQGNSMFPSC

SEQ ID NO: 172 - protein, 8 aa, Artificial Sequence
  Th epitope
CTKPTDGN

SEQ ID NO: 173 - protein, 8 aa, Artificial Sequence
  Th epitope
WASVRFSW

SEQ ID NO: 174 - protein, 9 aa, Artificial Sequence
  Th epitope
LLPIFFCLW

SEQ ID NO: 175 - protein, 20 aa, Artificial Sequence
  Th epitope
MDIDPYKEFGATVELLSFLP

SEQ ID NO: 176 - protein, 10 aa, Artificial Sequence
  Th epitope
FLPSDFFPSV

SEQ ID NO: 177 - protein, 20 aa, Artificial Sequence
  Th epitope
RDLLDTASALYREALESPEH

SEQ ID NO: 178 - protein, 20 aa, Artificial Sequence
  Th epitope
PHHTALRQAILCWGELMTLA

SEQ ID NO: 179 - protein, 15 aa, Artificial Sequence
  Th epitope
GRETVIEYLVSFGVW

SEQ ID NO: 180 - protein, 15 aa, Artificial Sequence
  Th epitope
EYLVSFGVWIRTPPA

SEQ ID NO: 181 - protein, 20 aa, Artificial Sequence
  Th epitope
VSFGVWIRTPPAYRPPNAPI

SEQ ID NO: 182 - protein, 10 aa, Artificial Sequence
  Th epitope
TVVRRRGRSP

SEQ ID NO: 183 - protein, 15 aa, Artificial Sequence
  Th epitope
VGPLTVNEKRRLKLI

SEQ ID NO: 184 - protein, 15 aa, Artificial Sequence
  Th epitope
RHYLHTLWKAGILYK

SEQ ID NO: 185 - protein, 15 aa, Artificial Sequence
  Th epitope
ESRLVVDFSQFSRGN

SEQ ID NO: 186 - protein, 15 aa, Artificial Sequence
  Th epitope
LQSLTNLLSSNLSWL

SEQ ID NO: 187 - protein, 15 aa, Artificial Sequence
  Th epitope
SSNLSWLSLDVSAAF

SEQ ID NO: 188 - protein, 15 aa, Artificial Sequence
  Th epitope
LHLYSHPIILGFRKI

SEQ ID NO: 189 - protein, 15 aa, Artificial Sequence
  Th epitope
KQCFRKLPVNRPIDW

SEQ ID NO: 190 - protein, 15 aa, Artificial Sequence
  Th epitope
LCQVFADATPTGWGL

SEQ ID NO: 191 - protein, 15 aa, Artificial Sequence
  Th epitope
AANWILRGTSFVYVP

SEQ ID NO: 192 - protein, 15 aa, Artificial Sequence
  Th epitope
EIRLKVFVLGGCRHK

SEQ ID NO: 193 - protein, 17 aa, Artificial Sequence
  Auxiliary part
  MISC_FEATURE (1)..(17): Xaa at position 17 is D-form alanine, Xaa at position 16 is 6-aminohexanoic acid.
GSHHHHHHGSDDDDKXX

SEQ ID NO: 194 - protein, 17 aa, Artificial Sequence
  Auxiliary part
  MISC_FEATURE (1)..(17): Xaa at position 1 is D-form alanine, Xaa at position 2 is 6-aminohexanoic acid.
XXGSHHHHHHGSDDDDK

SEQ ID NO: 195 - protein, 11 aa, Artificial Sequence
  Th epitope
KFVAAWTLKAA

SEQ ID NO: 196 - protein, 11 aa, Artificial Sequence
  Th epitope
KYVAAWTLKAA

SEQ ID NO: 197 - protein, 11 aa, Artificial Sequence
  Th epitope
KXVAAWTLKAA

SEQ ID NO: 198 - protein, 45 aa, Artificial Sequence; identical to SEQ ID NO: 108
  Unit peptide
  MISC_FEATURE (1)..(45): All Xaa are standard amino acid.

SEQ ID NO: 199 - protein, 45 aa, Artificial Sequence; identical to SEQ ID NO: 68
  Unit peptide
  MISC_FEATURE (1)..(45): All Xaa are standard amino acid.

SEQ ID NO: 200 - protein, 45 aa, Artificial Sequence; identical to SEQ ID NO: 69
  Unit peptide
  MISC_FEATURE (1)..(45): All Xaa are standard amino acid.

SEQ ID NO: 201 - protein, 50 aa, Artificial Sequence; identical to SEQ ID NO: 114
  Unit peptide
  MISC_FEATURE (1)..(50): All Xaa are standard amino acid.

SEQ ID NO: 202 - protein, 45 aa, Artificial Sequence; identical to SEQ ID NO: 84
  Unit peptide
  MISC_FEATURE (1)..(45): All Xaa are standard amino acid.

SEQ ID NO: 203 - protein, 45 aa, Artificial Sequence; identical to SEQ ID NO: 121
  Unit peptide
  MISC_FEATURE (1)..(45): All Xaa are standard amino acid.

SEQ ID NO: 204 - protein, 30 aa, Artificial Sequence; identical to SEQ ID NO: 56
  Unit peptide
  MISC_FEATURE (1)..(30): All Xaa are standard amino acid.

SEQ ID NO: 205 - protein, 26 aa, Artificial Sequence
  Unit peptide
  MISC_FEATURE (1)..(26): All Xaa are standard amino acid.
RNVPPIFNDVYWIAFKXVAAWTLKAA

SEQ ID NO: 206 - protein, 32 aa, Artificial Sequence; identical to SEQ ID NO: 67
  Unit peptide
  MISC_FEATURE (1)..(32): All Xaa are standard amino acid.

SEQ ID NO: 207 - protein, 43 aa, Artificial Sequence; identical to SEQ ID NO: 160
  Unit peptide
  MISC_FEATURE (1)..(43): All Xaa are standard amino acid.

SEQ ID NO: 208 - protein, 30 aa, Artificial Sequence; identical to SEQ ID NO: 161
  Unit peptide
  MISC_FEATURE (1)..(30): All Xaa are standard amino acid.

SEQ ID NO: 209 - protein, 45 aa, Artificial Sequence
  Unit peptide
  MISC_FEATURE (1)..(45): All Xaa are standard amino acid.
RNVPPIFNDVYWIAFXXKFVAAWTLKAAXXCRFRGLISLSQVYLS

SEQ ID NO: 210 - protein, 30 aa, Artificial Sequence
  Unit peptide
  MISC_FEATURE (1)..(30): All Xaa are standard amino acid.
RNVPPIFNDVYWIAFXXKFVAAWTLKAAXX

SEQ ID NO: 211 - protein, 43 aa, Artificial Sequence
  Unit peptide
  MISC_FEATURE (1)..(43): All Xaa are standard amino acid.
RNVPPIFNDVYWIAFXXKFVAAWTLKAACRFRGLISLSQVYLS

SEQ ID NO: 212 - protein, 30 aa, Artificial Sequence
  Unit peptide
  MISC_FEATURE (1)..(30): All Xaa are standard amino acid.
RNVPPIFNDVYWIAFXXKFVAAWTLKAACR

SEQ ID NO: 213 - protein, 23 aa, Artificial Sequence
  Unit peptide
RNVPPIFNDVYWIAFCTKPTDGN

SEQ ID NO: 214 - protein, 24 aa, Artificial Sequence
  Unit peptide
RNVPPIFNDVYWIAFLLPIFFCLW

SEQ ID NO: 215 - protein, 25 aa, Artificial Sequence
  Unit peptide
RNVPPIFNDVYWIAFFLPSDFFPSV

SEQ ID NO: 216 - protein, 55 aa, Artificial Sequence
  Unit peptide
  MISC_FEATURE (1)..(55): Xaa at position 22 and position 39 are D-form alanine, Xaa at position 21 and position 40 are 6-aminohexanoic acid.
KTTKQSFDLSVKAQYKKNKHXXWPEANQVGAGAFGPGFXXCRFRGLISLSQVYLS

SEQ ID NO: 217 - protein, 59 aa, Artificial Sequence
  Unit peptide
  MISC_FEATURE (1)..(59): Xaa at position 22 and position 43 are D-form alanine, Xaa at position 21 and position 44 are 6-aminohexanoic acid.
KTTKQSFDLSVKAQYKKNKHXXMDIDPYKEFGATVELLSFLPXXCRFRGLISLSQVYLS

SEQ ID NO: 218 - protein, 71 aa, Artificial Sequence
  Unit peptide
  MISC_FEATURE (1)..(71): Xaa at position 22 and position 55 are D-form alanine, Xaa at position 21 and position 56 are 6-aminohexanoic acid.
KTTKQSFDLSVKAQYKKNKHXXILMQYIKANSKFIGIPMGLPQSIALSSLMVAQXXCRFRGLISLSQVYLS

SEQ ID NO: 219 - protein, 36 aa, Artificial Sequence
  Unit peptide
RNVPPIFNDVYWIAFILMQYIKANSKFIGIHHHHHH

SEQ ID NO: 220 - protein, 41 aa, Artificial Sequence
  Unit peptide
RNVPPIFNDVYWIAFMDIDPYKEFGATVELLSFLPHHHHHH

SEQ ID NO: 221 - protein, 15 aa, Artificial Sequence
  B-cell epitope
RFRGLISLSQVYLDP

SEQ ID NO: 222 - protein, 15 aa, Artificial Sequence
  B-cell epitope
SVCGCPVGHHDVVGL

SEQ ID NO: 223 - protein, 21 aa, Artificial Sequence
  Th epitope
DIEKKIAKMEKASSVFNVVNS

SEQ ID NO: 224 - protein, 16 aa, Artificial Sequence
  Th epitope
YSGPLKAEIAQRLEDV

SEQ ID NO: 225 - protein, 11 aa, Artificial Sequence
  Th epitope
KXVKANTLKAA

SEQ ID NO: 226 - protein, 11 aa, Artificial Sequence
  Th epitope
KXVKANTLKAA

SEQ ID NO: 227 - protein, 11 aa, Artificial Sequence
  Th epitope
KXVKAWTLKAA

SEQ ID NO: 228 - protein, 11 aa, Artificial Sequence
  Th epitope
KXVKAWTLKAA

SEQ ID NO: 229 - protein, 11 aa, Artificial Sequence
  Th epitope
KXVWANTLKAA

SEQ ID NO: 230 - protein, 11 aa, Artificial Sequence
  Th epitope
KXVWANTLKAA

SEQ ID NO: 231 - protein, 11 aa, Artificial Sequence
  Th epitope
KXVWAYTLKAA

SEQ ID NO: 232 - protein, 11 aa, Artificial Sequence
  Th epitope
KXVWAVTLKAA

SEQ ID NO: 233 - protein, 11 aa, Artificial Sequence
  Th epitope
KXVYAWTLKAA

SEQ ID NO: 234 - protein, 11 aa, Artificial Sequence
  Th epitope
KXVYAWTLKAA

SEQ ID NO: 235 - protein, 11 aa, Artificial Sequence
  Th epitope
RXVRANTLKAA

SEQ ID NO: 236 - protein, 11 aa, Artificial Sequence
  Th epitope
KXVKAHTLKAA

SEQ ID NO: 237 - protein, 11 aa, Artificial Sequence
  Th epitope
KXVKAHTLKAA

SEQ ID NO: 238 - protein, 11 aa, Artificial Sequence
  Th epitope
KXVAANTLKAA

SEQ ID NO: 239 - protein, 11 aa, Artificial Sequence
  Th epitope
KXVAANTLKAA

SEQ ID NO: 240 - protein, 11 aa, Artificial Sequence
  Th epitope
KXVAAYTLKAA

SEQ ID NO: 241 - protein, 11 aa, Artificial Sequence
  Th epitope
KXVAAYTLKAA

SEQ ID NO: 242 - protein, 11 aa, Artificial Sequence
  Th epitope
KXVAAWTLKAA

SEQ ID NO: 243 - protein, 11 aa, Artificial Sequence
  Th epitope
KXVAAKTLKAA

SEQ ID NO: 244 - protein, 11 aa, Artificial Sequence
  Th epitope
KXVAAHTLKAA

SEQ ID NO: 245 - protein, 11 aa, Artificial Sequence
  Th epitope
KXVAAATLKAA

SEQ ID NO: 246 - protein, 11 aa, Artificial Sequence
  Th epitope
KXVAAWTLKAA

SEQ ID NO: 247 - protein, 11 aa, Artificial Sequence
  Th epitope
KXVMAATLKAA

SEQ ID NO: 248 - DNA, 135 bp, Artificial Sequence
  DNA encoding unit peptide
cgtaatgttcctcctatcttcaatgatgtttattggattgcattcnnnnnnaagnnngtggcagcttggaccctgaaggcagcannnnnntgccgtttccgtggactgatttccctgtcccaggtttatctgtcc

SEQ ID NO: 249 - DNA, 135 bp, Artificial Sequence
  DNA encoding unit peptide
cgtaatgttcctcctatcttcaatgatgtttattggattgcattcnnnnnnaagttcgtggcagcttggaccctgaaggcagcannnnnntgccgtttccgtggactgatttccctgtcccaggtttatctgtcc

SEQ ID NO: 250 - DNA, 135 bp, Artificial Sequence
  DNA encoding unit peptide
cgtaatgttcctcctatcttcaatgatgtttattggattgcattcnnnnnnaagtatgtggcagcttggaccctgaaggcagcannnnnntgccgtttccgtggactgatttccctgtcccaggtttatctgtcc

SEQ ID NO: 251 - DNA, 135 bp, Artificial Sequence
  DNA encoding unit peptide
cgtaatgttcctcctatcttcaatgatgtttattggattgcattcnnnnnnaagnnngtggcagcttggaccctgaaggcagcannnnnnggatcgcatcaccatcaccatcacggatccgatgatgatgacaag

SEQ ID NO: 252 - DNA, 135 bp, Artificial Sequence
  DNA encoding unit peptide
cgtaatgttcctcctatcttcaatgatgtttattggattgcattcnnnnnnaagttcgtggcagcttggaccctgaaggcagcannnnnnggatcgcatcaccatcaccatcacggatccgatgatgatgacaag

SEQ ID NO: 253 - DNA, 135 bp, Artificial Sequence
  DNA encoding unit peptide
cgtaatgttcctcctatcttcaatgatgtttattggattgcattcnnnnnnaagtatgtggcagcttggaccctgaaggcagcannnnnnggatcgcatcaccatcaccatcacggatccgatgatgatgacaag

SEQ ID NO: 254 - DNA, 135 bp, Artificial Sequence
  DNA encoding unit peptide
ggatcgcatcaccatcaccatcacggatccgatgatgatgacaagnnnnnnaagnnngtggcagcttggaccctgaaggcagcannnnnncgtaatgttcctcctatcttcaatgatgtttattggattgcattc

SEQ ID NO: 255 - DNA, 135 bp, Artificial Sequence
  DNA encoding unit peptide
ggatcgcatcaccatcaccatcacggatccgatgatgatgacaagnnnnnnaagttcgtggcagcttggaccctgaaggcagcannnnnncgtaatgttcctcctatcttcaatgatgtttattggattgcattc

SEQ ID NO: 256 - DNA, 135 bp, Artificial Sequence
  DNA encoding unit peptide
ggatcgcatcaccatcaccatcacggatccgatgatgatgacaagnnnnnnaagtatgtggcagcttggaccctgaaggcagcannnnnncgtaatgttcctcctatcttcaatgatgtttattggattgcattc

SEQ ID NO: 257 - DNA, 135 bp, Artificial Sequence
  DNA encoding unit peptide
aaaacgacaaagcaatcatttgatttaagtgtaaaagctcagtatnnnnnnaagnnngtggcagcttggaccctgaaggcagcannnnnntgccgtttccgtggactgatttccctgtcccaggtttatctgtcc

SEQ ID NO: 258 - DNA, 135 bp, Artificial Sequence
  DNA encoding unit peptide
aaaacgacaaagcaatcatttgatttaagtgtaaaagctcagtatnnnnnnaagttcgtggcagcttggaccctgaaggcagcannnnnntgccgtttccgtggactgatttccctgtcccaggtttatctgtcc

SEQ ID NO: 259 - DNA, 135 bp, Artificial Sequence
  DNA encoding unit peptide
aaaacgacaaagcaatcatttgatttaagtgtaaaagctcagtatnnnnnnaagtatgtggcagcttggaccctgaaggcagcannnnnntgccgtttccgtggactgatttccctgtcccaggtttatctgtcc

SEQ ID NO: 260 - DNA, 135 bp, Artificial Sequence
  DNA encoding unit peptide
cgtaatgttcctcctatcttcaatgatgtttattggattgcattctgccgtttccgtggactgatttccctgtcccaggtttatctgtccnnnnnnaagnnngtggcagcttggaccctgaaggcagcannnnnn

SEQ ID NO: 261 - DNA, 135 bp, Artificial Sequence
  DNA encoding unit peptide
cgtaatgttcctcctatcttcaatgatgtttattggattgcattctgccgtttccgtggactgatttccctgtcccaggtttatctgtccnnnnnnaagttcgtggcagcttggaccctgaaggcagcannnnnn

SEQ ID NO: 262 - DNA, 135 bp, Artificial Sequence
  DNA encoding unit peptide
cgtaatgttcctcctatcttcaatgatgtttattggattgcattctgccgtttccgtggactgatttccctgtcccaggtttatctgtccnnnnnnaagtatgtggcagcttggaccctgaaggcagcannnnnn

SEQ ID NO: 263 - DNA, 135 bp, Artificial Sequence
  DNA encoding unit peptide
cgtaatgttcctcctatcttcaatgatgtttattggattgcattcnnncctaagtatgtgaagcagaatacactgaagctggcaaccnnntgccgtttccgtggactgatttccctgtcccaggtttatctgtcc

SEQ ID NO: 264 - DNA, 90 bp, Artificial Sequence
  DNA encoding unit peptide
cgtaatgttcctcctatcttcaatgatgtttattggattgcattcnnnnnnaagnnngtggcagcttggaccctgaaggcagcannnnnn

SEQ ID NO: 265 - DNA, 90 bp, Artificial Sequence
  DNA encoding unit peptide
cgtaatgttcctcctatcttcaatgatgtttattggattgcattcnnnnnnaagttcgtggcagcttggaccctgaaggcagcannnnnn

SEQ ID NO: 266 - DNA, 90 bp, Artificial Sequence
  DNA encoding unit peptide
cgtaatgttcctcctatcttcaatgatgtttattggattgcattcnnnnnnaagtatgtggcagcttggaccctgaaggcagcannnnnn

SEQ ID NO: 267 - DNA, 78 bp, Artificial Sequence
  DNA encoding unit peptide
cgtaatgttcctcctatcttcaatgatgtttattggattgcattcaagnnngtggcagcttggaccctgaaggcagca

SEQ ID NO: 268 - DNA, 78 bp, Artificial Sequence
  DNA encoding unit peptide
cgtaatgttcctcctatcttcaatgatgtttattggattgcattcaagttcgtggcagcttggaccctgaaggcagca

SEQ ID NO: 269 - DNA, 78 bp, Artificial Sequence
  DNA encoding unit peptide
cgtaatgttcctcctatcttcaatgatgtttattggattgcattcaagtatgtggcagcttggaccctgaaggcagca

SEQ ID NO: 270 - DNA, 96 bp, Artificial Sequence
  DNA encoding unit peptide
cgtaatgttcctcctatcttcaatgatgtttattggattgcattcaagnnngtggcagcttggaccctgaaggcagcacatcaccatcaccatcac

SEQ ID NO: 271 - DNA, 96 bp, Artificial Sequence
  DNA encoding unit peptide
cgtaatgttcctcctatcttcaatgatgtttattggattgcattcaagttcgtggcagcttggaccctgaaggcagcacatcaccatcaccatcac

SEQ ID NO: 272 - DNA, 96 bp, Artificial Sequence
  DNA encoding unit peptide
cgtaatgttcctcctatcttcaatgatgtttattggattgcattcaagtatgtggcagcttggaccctgaaggcagcacatcaccatcaccatcac

SEQ ID NO: 273 - DNA, 129 bp, Artificial Sequence
  DNA encoding unit peptide
cgtaatgttcctcctatcttcaatgatgtttattggattgcattcnnnnnnaagnnngtggcagcttggaccctgaaggcagcatgccgtttccgtggactgatttccctgtcccaggtttatctgtcc

SEQ ID NO: 274 - DNA, 129 bp, Artificial Sequence
  DNA encoding unit peptide
cgtaatgttcctcctatcttcaatgatgtttattggattgcattcnnnnnnaagttcgtggcagcttggaccctgaaggcagcatgccgtttccgtggactgatttccctgtcccaggtttatctgtcc

SEQ ID NO: 275 - DNA, 129 bp, Artificial Sequence
  DNA encoding unit peptide
cgtaatgttcctcctatcttcaatgatgtttattggattgcattcnnnnnnaagtatgtggcagcttggaccctgaaggcagcatgccgtttccgtggactgatttccctgtcccaggtttatctgtcc

SEQ ID NO: 276 - DNA, 90 bp, Artificial Sequence
  DNA encoding unit peptide
cgtaatgttcctcctatcttcaatgatgtttattggattgcattcnnnnnnaagnnngtggcagcttggaccctgaaggcagcatgccgt

SEQ ID NO: 277 - DNA, 90 bp, Artificial Sequence
  DNA encoding unit peptide
cgtaatgttcctcctatcttcaatgatgtttattggattgcattcnnnnnnaagttcgtggcagcttggaccctgaaggcagcatgccgt

SEQ ID NO: 278 - DNA, 90 bp, Artificial Sequence
  DNA encoding unit peptide
cgtaatgttcctcctatcttcaatgatgtttattggattgcattcnnnnnnaagtatgtggcagcttggaccctgaaggcagcatgccgt

SEQ ID NO: 279 - RNA, 135 nt, Artificial Sequence
  RNA encoding unit peptide
cguaauguuccuccuaucuucaaugauguuuauuggauugcauucnnnnnnaagnnnguggcagcuuggacccugaaggcagcannnnnnugccguuuccguggacugauuucccugucccagguuuaucugucc

SEQ ID NO: 280 - RNA, 135 nt, Artificial Sequence
  RNA encoding unit peptide
cguaauguuccuccuaucuucaaugauguuuauuggauugcauucnnnnnnaaguucguggcagcuuggacccugaaggcagcannnnnnugccguuuccguggacugauuucccugucccagguuuaucugucc

SEQ ID NO: 281 - RNA, 135 nt, Artificial Sequence
  RNA encoding unit peptide
cguaauguuccuccuaucuucaaugauguuuauuggauugcauucnnnnnnaaguauguggcagcuuggacccugaaggcagcannnnnnugccguuuccguggacugauuucccugucccagguuuaucugucc

SEQ ID NO: 282 - RNA, 135 nt, Artificial Sequence
  RNA encoding unit peptide
cguaauguuccuccuaucuucaaugauguuuauuggauugcauucnnnnnnaagnnnguggcagcuuggacccugaaggcagcannnnnnggaucgcaucaccaucaccaucacggauccgaugaugaugacaag

SEQ ID NO: 283 - RNA, 135 nt, Artificial Sequence
  RNA encoding unit peptide
cguaauguuccuccuaucuucaaugauguuuauuggauugcauucnnnnnnaaguucguggcagcuuggacccugaaggcagcannnnnnggaucgcaucaccaucaccaucacggauccgaugaugaugacaag

SEQ ID NO: 284 - RNA, 135 nt, Artificial Sequence
  RNA encoding unit peptide
cguaauguuccuccuaucuucaaugauguuuauuggauugcauucnnnnnnaaguauguggcagcuuggacccugaaggcagcannnnnnggaucgcaucaccaucaccaucacggauccgaugaugaugacaag

SEQ ID NO: 285 - RNA, 135 nt, Artificial Sequence
  RNA encoding unit peptide
ggaucgcaucaccaucaccaucacggauccgaugaugaugacaagnnnnnnaagnnnguggcagcuuggacccugaaggcagcannnnnncguaauguuccuccuaucuucaaugauguuuauuggauugcauuc

SEQ ID NO: 286 - RNA, 135 nt, Artificial Sequence
  RNA encoding unit peptide
ggaucgcaucaccaucaccaucacggauccgaugaugaugacaagnnnnnnaaguucguggcagcuuggacccugaaggcagcannnnnncguaauguuccuccuaucuucaaugauguuuauuggauugcauuc

SEQ ID NO: 287 - RNA, 135 nt, Artificial Sequence
  RNA encoding unit peptide
ggaucgcaucaccaucaccaucacggauccgaugaugaugacaagnnnnnnaaguauguggcagcuuggacccugaaggcagcannnnnncguaauguuccuccuaucuucaaugauguuuauuggauugcauuc

SEQ ID NO: 288 - RNA, 135 nt, Artificial Sequence
  RNA encoding unit peptide
aaaacgacaaagcaaucauuugauuuaaguguaaaagcucaguaunnnnnnaagnnnguggcagcuuggacccugaaggcagcannnnnnugccguuuccguggacugauuucccugucccagguuuaucugucc

SEQ ID NO: 289 - RNA, 135 nt, Artificial Sequence
  RNA encoding unit peptide
aaaacgacaaagcaaucauuugauuuaaguguaaaagcucaguaunnnnnnaaguucguggcagcuuggacccugaaggcagcannnnnnugccguuuccguggacugauuucccugucccagguuuaucugucc

SEQ ID NO: 290 - RNA, 135 nt, Artificial Sequence
  RNA encoding unit peptide
aaaacgacaaagcaaucauuugauuuaaguguaaaagcucaguaunnnnnnaaguauguggcagcuuggacccugaaggcagcannnnnnugccguuuccguggacugauuucccugucccagguuuaucugucc

SEQ ID NO: 291 - RNA, 135 nt, Artificial Sequence
  RNA encoding unit peptide
cguaauguuccuccuaucuucaaugauguuuauuggauugcauucugccguuuccguggacugauuucccugucccagguuuaucuguccnnnnnnaagnnnguggcagcuuggacccugaaggcagcannnnnn

SEQ ID NO: 292 - RNA, 135 nt, Artificial Sequence
  RNA encoding unit peptide
cguaauguuccuccuaucuucaaugauguuuauuggauugcauucugccguuuccguggacugauuucccugucccagguuuaucuguccnnnnnnaaguucguggcagcuuggacccugaaggcagcannnnnn

SEQ ID NO: 293 - RNA, 135 nt, Artificial Sequence
  RNA encoding unit peptide
cguaauguuccuccuaucuucaaugauguuuauuggauugcauucugccguuuccguggacugauuucccugucccagguuuaucuguccnnnnnnaaguauguggcagcuuggacccugaaggcagcannnnnn

SEQ ID NO: 294 - RNA, 135 nt, Artificial Sequence
  RNA encoding unit peptide
cguaauguuccuccuaucuucaaugauguuuauuggauugcauucnnnccuaaguaugugaagcagaauacacugaagcuggcaaccnnnugccguuuccguggacugauuucccugucccagguuuaucugucc

SEQ ID NO: 295 - RNA, 90 nt, Artificial Sequence
  RNA encoding unit peptide
cguaauguuccuccuaucuucaaugauguuuauuggauugcauucnnnnnnaagnnnguggcagcuuggacccugaaggcagcannnnnn

SEQ ID NO: 296 - RNA, 90 nt, Artificial Sequence
  RNA encoding unit peptide
cguaauguuccuccuaucuucaaugauguuuauuggauugcauucnnnnnnaaguucguggcagcuuggacccugaaggcagcannnnnn

SEQ ID NO: 297 - RNA, 90 nt, Artificial Sequence
  RNA encoding unit peptide
cguaauguuccuccuaucuucaaugauguuuauuggauugcauucnnnnnnaaguauguggcagcuuggacccugaaggcagcannnnnn

SEQ ID NO: 298 - RNA, 78 nt, Artificial Sequence
  RNA encoding unit peptide
cguaauguuccuccuaucuucaaugauguuuauuggauugcauucaagnnnguggcagcuuggacccugaaggcagca

SEQ ID NO: 299 - RNA, 78 nt, Artificial Sequence
  RNA encoding unit peptide
cguaauguuccuccuaucuucaaugauguuuauuggauugcauucaaguucguggcagcuuggacccugaaggcagca

SEQ ID NO: 300 - RNA, 78 nt, Artificial Sequence
  RNA encoding unit peptide
cguaauguuccuccuaucuucaaugauguuuauuggauugcauucaaguauguggcagcuuggacccugaaggcagca

SEQ ID NO: 301 - RNA, 96 nt, Artificial Sequence
  RNA encoding unit peptide
cguaauguuccuccuaucuucaaugauguuuauuggauugcauucaagnnnguggcagcuuggacccugaaggcagcacaucaccaucaccaucac

SEQ ID NO: 302 - RNA, 96 nt, Artificial Sequence
  RNA encoding unit peptide
cguaauguuccuccuaucuucaaugauguuuauuggauugcauucaaguucguggcagcuuggacccugaaggcagcacaucaccaucaccaucac

SEQ ID NO: 303 - RNA, 96 nt, Artificial Sequence
  RNA encoding unit peptide
cguaauguuccuccuaucuucaaugauguuuauuggauugcauucaaguauguggcagcuuggacccugaaggcagcacaucaccaucaccaucac

SEQ ID NO: 304 - RNA, 129 nt, Artificial Sequence
  RNA encoding unit peptide
cguaauguuccuccuaucuucaaugauguuuauuggauugcauucnnnnnnaagnnnguggcagcuuggacccugaaggcagcaugccguuuccguggacugauuucccugucccagguuuaucugucc

SEQ ID NO: 305 - RNA, 129 nt, Artificial Sequence
  RNA encoding unit peptide
cguaauguuccuccuaucuucaaugauguuuauuggauugcauucnnnnnnaaguucguggcagcuuggacccugaaggcagcaugccguuuccguggacugauuucccugucccagguuuaucugucc

SEQ ID NO: 306 - RNA, 129 nt, Artificial Sequence
  RNA encoding unit peptide
cguaauguuccuccuaucuucaaugauguuuauuggauugcauucnnnnnnaaguauguggcagcuuggacccugaaggcagcaugccguuuccguggacugauuucccugucccagguuuaucugucc

SEQ ID NO: 307 - RNA, 90 nt, Artificial Sequence
  RNA encoding unit peptide
cguaauguuccuccuaucuucaaugauguuuauuggauugcauucnnnnnnaagnnnguggcagcuuggacccugaaggcagcaugccgu

SEQ ID NO: 308 - RNA, 90 nt, Artificial Sequence
  RNA encoding unit peptide
cguaauguuccuccuaucuucaaugauguuuauuggauugcauucnnnnnnaaguucguggcagcuuggacccugaaggcagcaugccgu

SEQ ID NO: 309 - RNA, 90 nt, Artificial Sequence
  RNA encoding unit peptide
cguaauguuccuccuaucuucaaugauguuuauuggauugcauucnnnnnnaaguauguggcagcuuggacccugaaggcagcaugccgu